European Patent Application EP 4 814 010 A1, published September 30, 2026. Title: 靶向IL-11的抗原结合蛋白. Applicant: 上海华奥泰生物药业股份有限公司. The sequence listing filed with the application follows.

SEQUENCE LISTING (16 sequences)

SEQ ID NO: 1 - protein, 5 aa, synthetic construct
  REGION 1..5: note = 700068 CDR1 700077 CDR1
IYTMA

SEQ ID NO: 2 - protein, 16 aa, synthetic construct
  REGION 1..16: note = 700068 CDR2 700077 CDR2
LSTNRGATDYADFVKG

SEQ ID NO: 3 - protein, 12 aa, synthetic construct
  REGION 1..12: note = 700068 CDR3700077 CDR3
VASSWSTGFVAS

SEQ ID NO: 4 - protein, 30 aa, synthetic construct
  REGION 1..30: note = 700068 FR1 700077 FR1
QVQLVESGGGLVQPGGSLRLSCAASGSIAS

SEQ ID NO: 5 - protein, 14 aa, synthetic construct
  REGION 1..14: note = 700068 FR2 700077 FR2
WYRQAPGKQRELVA

SEQ ID NO: 6 - protein, 32 aa, synthetic construct
  REGION 1..32: note = 700068 FR3 700077 FR3
RFTISRDNAENTMYLQMNSLKPEDTAVYYCNG

SEQ ID NO: 7 - protein, 11 aa, synthetic construct
  REGION 1..11: note = 700068 FR4 700077 FR4
WGQGTQVTVSS

SEQ ID NO: 8 - protein, 233 aa, synthetic construct
  REGION 1..233: note = 700068 FC
GSEPKSCDKTHTCPPCPAPEAAGGPSVFLFPPKPKDTLMISRTPEVTCVVVDVSHEDPEVKFNWYVDGVEVHNAKTKPREEQYNSTYRVVSVLTVLHQDWLNGKEYKCKVSNKALPAPIEKTISKAKGQPREPQVYTLPPSREEMTKNQVSLTCLVKGFYPSDIAVEWESNGQPENNYKTTPPVLDSDGSFFLYSKLTVDKSRWQQGNVFSCSVMHEALHNHYTQKSLSLSPG

SEQ ID NO: 9 - protein, 231 aa, synthetic construct
  REGION 1..231: note = 700077 Fc
EPKSSDKTHTCPPCPAPEAAGGPSVFLFPPKPKDTLMISRTPEVTCVVVDVSHEDPEVKFNWYVDGVEVHNAKTKPREEQYNSTYRVVSVLTVLHQDWLNGKEYKCKVSNKALPAPIEKTISKAKGQPREPQVYTLPPSREEMTKNQVSLTCLVKGFYPSDIAVEWESNGQPENNYKTTPPVLDSDGSFFLYSKLTVDKSRWQQGNVFSCSVMHEALHNHYTQKSLSLSPG

SEQ ID NO: 10 - protein, 120 aa, synthetic construct
  REGION 1..120: note = 700068 VHH 70077VHH
QVQLVESGGGLVQPGGSLRLSCAASGSIASIYTMAWYRQAPGKQRELVALSTNRGATDYADFVKGRFTISRDNAENTMYLQMNSLKPEDTAVYYCNGVASSWSTGFVASWGQGTQVTVSS

SEQ ID NO: 11 - DNA, 1059 bp, synthetic construct
  misc_feature 1..1059: note = 400208 plasmid
  source 1..1059: mol_type = other DNA
caagtgcagctcgtggagagcggcggaggactcgtgcaacctggcggctccctgagactgagctgcgccgctagcggcagcatcgctagcatctacaccatggcctggtacagacaagcccctggcaagcagagagagctggtggccctgagcaccaacagaggcgccaccgactacgccgacttcgtgaagggcagattcaccatcagcagagacaacgccgagaacaccatgtacctgcagatgaacagcctgaagcctgaggacaccgccgtgtactactgcaacggcgtggctagcagctggagcaccggcttcgtggctagctggggccaaggcacccaagtgaccgtgagcagcggatccgagcccaaatcttgtgacaaaactcacacatgcccaccgtgcccagcacctgaagccgctgggggaccgtcagtcttcctcttccccccaaaacccaaggacaccctcatgatctcccggacccctgaggtcacatgcgtggtggtggacgtgagccacgaagaccctgaggtcaagttcaactggtacgtggacggcgtggaggtgcataatgccaagacaaagccgcgggaggagcagtacaacagcacgtaccgtgtggtcagcgtcctcaccgtcctgcaccaggactggctgaatggcaaggagtacaagtgcaaggtctccaacaaagccctcccagcccccatcgagaaaaccatctccaaagccaaagggcagccccgagaaccacaggtgtacaccctgcccccatcccgcgaggagatgaccaagaaccaggtaagtttgacctgcctggtcaaaggcttctatcccagcgacatcgccgtggagtgggagagcaatgggcagccggagaacaactacaagaccacgcctcccgtgctggactccgacggctccttcttcctctatagcaagctcaccgtggacaagagcaggtggcagcaggggaacgtcttctcatgctccgtgatgcatgaggctctgcacaaccactacacgcagaagagcctctccctgtctccgggt

SEQ ID NO: 12 - DNA, 1053 bp, synthetic construct
  misc_feature 1..1053: note = 400231 plasmid
  source 1..1053: mol_type = other DNA
caagtgcagctcgtggagagcggcggaggactcgtgcaacctggcggctccctgagactgagctgcgccgctagcggcagcatcgctagcatctacaccatggcctggtacagacaagcccctggcaagcagagagagctggtggccctgagcaccaacagaggcgccaccgactacgccgacttcgtgaagggcagattcaccatcagcagagacaacgccgagaacaccatgtacctgcagatgaacagcctgaagcctgaggacaccgccgtgtactactgcaacggcgtggctagcagctggagcaccggcttcgtggctagctggggccaaggcacccaagtgaccgtgagcagcgagcccaaatcttctgacaaaactcacacatgcccaccgtgcccagcacctgaagccgctgggggaccgtcagtcttcctcttccccccaaaacccaaggacaccctcatgatctcccggacccctgaggtcacatgcgtggtggtggacgtgagccacgaagaccctgaggtcaagttcaactggtacgtggacggcgtggaggtgcataatgccaagacaaagccgcgggaggagcagtacaacagcacgtaccgtgtggtcagcgtcctcaccgtcctgcaccaggactggctgaatggcaaggagtacaagtgcaaggtctccaacaaagccctcccagcccccatcgagaaaaccatctccaaagccaaagggcagccccgagaaccacaggtgtacaccctgcccccatcccgcgaggagatgaccaagaaccaggtaagtttgacctgcctggtcaaaggcttctatcccagcgacatcgccgtggagtgggagagcaatgggcagccggagaacaactacaagaccacgcctcccgtgctggactccgacggctccttcttcctctatagcaagctcaccgtggacaagagcaggtggcagcaggggaacgtcttctcatgctccgtgatgcatgaggctctgcacaaccactacacgcagaagagcctctccctgtctccgggt

SEQ ID NO: 13 - DNA, 38 bp, synthetic construct
  misc_feature 1..38: note = Primer-400208-F
  source 1..38: mol_type = other DNA
gagcagcgagcccaaatcttctgacaaaactcacacat

SEQ ID NO: 14 - DNA, 35 bp, synthetic construct
  misc_feature 1..35: note = Primer-400208-R
  source 1..35: mol_type = other DNA
cagaagatttgggctcgctgctcacggtcacttgg

SEQ ID NO: 15 - DNA, 38 bp, synthetic construct
  misc_feature 1..38: note = Primer-400216-F
  source 1..38: mol_type = other DNA
accgtccttgacacgaagcttgccgccaccatgggatg

SEQ ID NO: 16 - DNA, 47 bp, synthetic construct
  misc_feature 1..47: note = Primer-400216-R
  source 1..47: mol_type = other DNA
gctgattatgatcaatgaattctcaacccggagacagggagaggctc